European Patent Application EP 4 810 055 A1, published September 23, 2026. Title: 탈수초 질환 치료용 펩타이드 및 이의 용도. Applicant: (주)카인사이언스. Application KR. The sequence listing filed with the application follows.

SEQUENCE LISTING (1 sequence)

SEQ ID NO: 1 - protein, 9 aa, synthetic construct
PSPPSPPSP